European Patent Application EP 4 141 115 A1, published March 1, 2023. Title: Method of Detecting an Nucleic acid and Oligonucleotide Probe. Applicant: Nicca Chemicall  Co., Ltd. University of Fukui. The sequence listing filed with the application follows.

SEQUENCE LISTING (36 sequences)

SEQ ID NO: 1 - DNA, 34 bp, Artificial sequence
  Probe
tgctactaccaccaagatctgcacctgcggcggc

SEQ ID NO: 2 - DNA, 25 bp, Artificial sequence
  Probe
gctactaccaccaagatctgcacct

SEQ ID NO: 3 - DNA, 17 bp, Artificial sequence
  Probe
tgctactaccaccaaga

SEQ ID NO: 4 - DNA, 34 bp, Artificial sequence
  Probe
  modified_base (24)..(24): n is a photocrosslinkable functional group
  misc_feature (24)..(24): n is a, c, g, or t
tgctactaccaccaagatctgcanctgcggcggc

SEQ ID NO: 5 - DNA, 25 bp, Artificial sequence
  Probe
  modified_base (23)..(23): n is a photocrosslinkable functional group
  misc_feature (23)..(23): n is a, c, g, or t
gctactaccaccaagatctgcanct

SEQ ID NO: 6 - DNA, 17 bp, Artificial sequence
  Probe
  modified_base (15)..(15): n is a photocrosslinkable functional group
  misc_feature (15)..(15): n is a, c, g, or t
tgctactaccaccanga

SEQ ID NO: 7 - DNA, 20 bp, Artificial sequence
  Probe
  modified_base (18)..(18): n is a photocrosslinkable functional group
  misc_feature (18)..(18): n is a, c, g, or t
gagcgcggtctccaccanct

SEQ ID NO: 8 - DNA, 20 bp, Artificial sequence
  Probe
  modified_base (18)..(18): n is a photocrosslinkable functional group
  misc_feature (18)..(18): n is a, c, g, or t
gctgtgggaataccccangg

SEQ ID NO: 9 - DNA, 20 bp, Artificial sequence
  Probe
  modified_base (18)..(18): n is a photocrosslinkable functional group
  misc_feature (18)..(18): n is a, c, g, or t
cctccctagcttgattantc

SEQ ID NO: 10 - DNA, 20 bp, Artificial sequence
  Probe
  modified_base (18)..(18): n is a photocrosslinkable functional group
  misc_feature (18)..(18): n is a, c, g, or t
cacataactgagggggangg

SEQ ID NO: 11 - DNA, 20 bp, Artificial sequence
  Probe
  modified_base (18)..(18): n is a photocrosslinkable functional group
  misc_feature (18)..(18): n is a, c, g, or t
cggccacagtcgcatcangg

SEQ ID NO: 12 - DNA, 20 bp, Artificial sequence
  Probe
  modified_base (18)..(18): n is a photocrosslinkable functional group
  misc_feature (18)..(18): n is a, c, g, or t
ggatcttcagcgtcacancg

SEQ ID NO: 13 - DNA, 20 bp, Artificial sequence
  Probe
  modified_base (18)..(18): n is a photocrosslinkable functional group
  misc_feature (18)..(18): n is a, c, g, or t
cgcaggcaagtcttccanct

SEQ ID NO: 14 - DNA, 20 bp, Artificial sequence
  Probe
  modified_base (18)..(18): n is  a ribonucleosides with photocrosslinkable functional group
  misc_feature (18)..(18): n is a, c, g, or t
acggtggcgtggttccantg

SEQ ID NO: 15 - DNA, 20 bp, Artificial sequence
  Probe
  modified_base (18)..(18): n is a photocrosslinkable functional group
  misc_feature (18)..(18): n is a, c, g, or t
gcagttcctttaaggcantg

SEQ ID NO: 16 - DNA, 20 bp, Artificial sequence
  Probe
  modified_base (18)..(18): n is a photocrosslinkable functional group
  misc_feature (18)..(18): n is a, c, g, or t
taatgtgctctggttcantt

SEQ ID NO: 17 - DNA, 20 bp, Artificial sequence
  Probe
  modified_base (18)..(18): n is a photocrosslinkable functional group
  misc_feature (18)..(18): n is a, c, g, or t
ctctgggagagagggcantc

SEQ ID NO: 18 - DNA, 20 bp, Artificial sequence
  Probe
  modified_base (18)..(18): n is a photocrosslinkable functional group
  misc_feature (18)..(18): n is a, c, g, or t
tatttacaatggatgaantc

SEQ ID NO: 19 - DNA, 20 bp, Artificial sequence
  Probe
  modified_base (18)..(18): n is a photocrosslinkable functional group
  misc_feature (18)..(18): n is a, c, g, or t
gacacattggcatagtangt

SEQ ID NO: 20 - DNA, 20 bp, Artificial sequence
  Probe
  modified_base (18)..(18): n is a photocrosslinkable functional group
  misc_feature (18)..(18): n is a, c, g, or t
ctcccaaactcctggcantt

SEQ ID NO: 21 - DNA, 20 bp, Artificial sequence
  Probe
  modified_base (18)..(18): n is a photocrosslinkable functional group
  misc_feature (18)..(18): n is a, c, g, or t
acttttatcttcttatantt

SEQ ID NO: 22 - DNA, 20 bp, Artificial sequence
  Probe
  modified_base (18)..(18): n is a photocrosslinkable functional group
  misc_feature (18)..(18): n is a, c, g, or t
gaacacaatagtctgaangg

SEQ ID NO: 23 - DNA, 20 bp, Artificial sequence
  Probe
  modified_base (18)..(18): n is a photocrosslinkable functional group
  misc_feature (18)..(18): n is a, c, g, or t
catatttggtaaatgcantg

SEQ ID NO: 24 - DNA, 20 bp, Artificial sequence
  Probe
  modified_base (18)..(18): n is a photocrosslinkable functional group
  misc_feature (18)..(18): n is a, c, g, or t
tttgcccagggatgccanct

SEQ ID NO: 25 - DNA, 20 bp, Artificial sequence
  Probe
  modified_base (18)..(18): n is a photocrosslinkable functional group
  misc_feature (18)..(18): n is a, c, g, or t
atttggctatgaggagantg

SEQ ID NO: 26 - DNA, 20 bp, Artificial sequence
  Probe
  modified_base (18)..(18): n is a photocrosslinkable functional group
  misc_feature (18)..(18): n is a, c, g, or t
ggtttcggattggagtantg

SEQ ID NO: 27 - DNA, 20 bp, Artificial sequence
  Probe
  modified_base (18)..(18): n is a photocrosslinkable functional group
  misc_feature (18)..(18): n is a, c, g, or t
gctcatgatgggctggantg

SEQ ID NO: 28 - DNA, 20 bp, Artificial sequence
  Probe
  modified_base (18)..(18): n is a photocrosslinkable functional group
  misc_feature (18)..(18): n is a, c, g, or t
tgagctgcggtgagaganga

SEQ ID NO: 29 - DNA, 20 bp, Artificial sequence
  Probe
  modified_base (18)..(18): n is a photocrosslinkable functional group
  misc_feature (18)..(18): n is a, c, g, or t
ctatttgctgcctgacangc

SEQ ID NO: 30 - DNA, 20 bp, Artificial sequence
  Probe
  modified_base (18)..(18): n is a photocrosslinkable functional group
  misc_feature (18)..(18): n is a, c, g, or t
tatctgttggtttatcanat

SEQ ID NO: 31 - DNA, 20 bp, Artificial sequence
  Probe
  modified_base (18)..(18): n is a photocrosslinkable functional group
  misc_feature (18)..(18): n is a, c, g, or t
atgctggtgagccaggantc

SEQ ID NO: 32 - DNA, 20 bp, Artificial sequence
  Probe
  modified_base (18)..(18): n is a photocrosslinkable functional group
  misc_feature (18)..(18): n is a, c, g, or t
gggtgggtggttcaaganct

SEQ ID NO: 33 - DNA, 24 bp, Artificial Sequence
  probe
  modified_base (22)..(22): n is a photocrosslinkable functional group
  misc_feature (22)..(22): n is a, c, g, or t
gtccacacaggagtgggtgcantt

SEQ ID NO: 34 - DNA, 24 bp, Artificial Sequence
  probe
  modified_base (22)..(22): n is a photocrosslinkable functional group
  misc_feature (22)..(22): n is a, c, g, or t
cgtcagagggctggctctctgntc

SEQ ID NO: 35 - DNA, 20 bp, Artificial sequence
  Probe
  modified_base (18)..(18): n is a photocrosslinkable functional group
  misc_feature (18)..(18): n is a, c, g, or t
gtctcctccctagcaaancc

SEQ ID NO: 36 - DNA, 20 bp, Artificial sequence
  Probe
  modified_base (18)..(18): n is a photocrosslinkable functional group
  misc_feature (18)..(18): n is a, c, g, or t
gtctgggaagacaaccanag